European Patent Specification EP 3 971 217 B1, published December 27, 2023. Title: Method for increasing yield of sprayed corn bran in corn wet milling process. Applicant: Novozymes. The sequence listing filed with the application follows.

SEQUENCE LISTING (2 sequences)

SEQ ID NO: 1 - protein, 319 aa, Aspergillus Niger
MVQIKVAALAMLFASQVLSEPIEPRQASVSIDTKFKAHGKKYLGNIGDQYTLTKNSKTPAIIKADFGALTPENSMKWDATEPSRGQFSFSGSDYLVNFAQSNNKLIRGHTLVWHSQLPSWVQSITDKNTLIEVMENHITTVMQHYKGKIYAWDVVNEIFNEDGSLRDSVFYKVIGEDYVRIAFETARAADPNAKLYINDYNLDSASYPKLTGMVSHVKKWIAAGIPIDGIGSQTHLSAALNALAGAGTKEIAVTELDIAGASSTDYVEVVEACLNQPKCIGITVWGVADPDSWRSSSTPLLFDSNYNPKPAYTAIANAL

SEQ ID NO: 2 - protein, 332 aa, Aspergillus Niger
MKFFNAKGSLLSSGIYLIALTPFVNAKCSLPSSYSWSSTDALATPKSGWTALKDFTDVVSDGKHIVYASTTDEAGNYGSMTFGAFSEWSNMASASQTATPFNAVAPTLFYFKPKSIWVLAYQWGSSTFTYRTSQDPTNVNGWSSEQALFTGKLSDSSTGAIDQTVIGDDTNMYLFFAGDNGKIYRSSMSIDEFPGSFGSQYEEILSGATNDLFEAVQVYTVDGGEGNSKYLMIVEAIGSTGHRYFRSFTASSLGGEWTAQAASEDKPFAGKANSGATWTEDISHGDLVRNNPDQTMTVDPCNLQLLYQGHDPNSSGDYNLLPWKPGVLTLKQ